European Patent Specification EP 3 649 150 B1, published June 26, 2024. Title: ROR1 CAR T-CELLS. Applicant: UCL Business PLC. The sequence listing filed with the application follows.

SEQUENCE LISTING (62 sequences)

SEQ ID NO: 1 - protein, 15 aa, Artificial sequence
  Linker
GGGGSGGGGSGGGGS

SEQ ID NO: 2 - protein, 5 aa, Artificial sequence
  Linker
GGGGS

SEQ ID NO: 3 - protein, 107 aa, Rattus norvegicus
DIQMTQSPSFLSASVGDRVTINCKASQNIDRYLNWYQQKLGEAPKRLLYNTNKLQTGIPSRFSGSGSATDFTLTISSLQPEDFATYFCLQYNSLPLTFGSGTKLEIK

SEQ ID NO: 4 - protein, 107 aa, Artificial sequence
  Humanised light chain variable region
DIQMTQSPSSLSASVGDRVTITCKASQNIDRYLNWYQQKPGKAPKRLIYNTNKLQTGVPSRFSGSGSGTEFTLTISSLQPEDFATYYCLQYNSLPLTFGQGTKLEIK

SEQ ID NO: 5 - protein, 107 aa, Artificial sequence
  Humanised light chain variable region
DIQMTQSPSSLSASVGDRVTITCKASQNIDRYLNWFQQKPGKAPKSLIYNTNKLQTGVPSKFSGSGSGTDFTLTISSLQPEDFATYYCLQYNSLPLTFGQGTRLEIK

SEQ ID NO: 6 - protein, 107 aa, Artificial sequence
  Humanised light chain variable region
DIQMTQSPSSLSASVGDRVTITCKASQNIDRYLNWYQQKPGKAPKLLIYNTNKLQTGVPSRFSGSGSGTDFTLTISSLQPEDFATYYCLQYNSLPLTFGQGTKLEIK

SEQ ID NO: 7 - protein, 107 aa, Artificial sequence
  Humanised light chain variable region
DIQLTQSPSFLSASVGDRVTITCKASQNIDRYLNWYQQKPGKAPKLLIYNTNKLQTGVPSRFSGSGSGTEFTLTISSLQPEDFATYYCLQYNSLPLTFGQGTKLEIK

SEQ ID NO: 8 - protein, 107 aa, Artificial sequence
  Humanised light chain variable region
DIQMTQSPSTLSASVGDRVTITCKASQNIDRYLNWYQQKPGKAPKLLIYNTNKLQTGVPSRFSGSGSGTEFTLTISSLQPDDFATYYCLQYNSLPLTFGQGTKLEIK

SEQ ID NO: 9 - protein, 117 aa, Rattus norvegicus
EVQLVESGGGLVQPGRSLKLSCAASGFIFSEHNMAWVRQAPKKGLEWVATISDDGRNTYYRDSMRGRFTISRENARSTLYLQLDSLRSEDTATYYCASHRYNLFDSWGQGVMVTVSS

SEQ ID NO: 10 - protein, 117 aa, Artificial sequence
  Humanised heavy chain variable region
QVQLVESGGGVVQPGRSLRLSCAASGFIFSEHNMAWVRQAPGKGLEWVATISDDGRNTYYRDSMRGRFTISRDNSKNTLYLQMNSLRAEDTAVYYCTSHRYNLFDSWGQGTMVTVSS

SEQ ID NO: 11 - protein, 117 aa, Artificial sequence
  Humanised heavy chain variable region
EVQLVESGGGLVQPGGSLRLSCAASGFIFSEHNMAWVRQAPGKGLEWVSTISDDGRNTYYRDSMRGRFTISRDNSKNTLYLQMNSLRAEDTAVYYCAKHRYNLFDSWGQGTLVTVSS

SEQ ID NO: 12 - protein, 117 aa, Artificial sequence
  Humanised heavy chain variable region
EVQLVESGGGLVQPGGSLRLSCAASGFIFSEHNMAWVRQAPGKGLEWVATISDDGRNTYYRDSMRGRFTISRDNAKNSLYLQMNSLRAEDTAVYYCARHRYNLFDSWGQGTMVTVSS

SEQ ID NO: 13 - protein, 117 aa, Artificial sequence
  Humanised heavy chain variable region
EVQLVESGGGLVQPGGSLRLSCAASGFIFSEHNMAWVRQAPGKGLVWVSTISDDGRNTYYRDSMRGRFTISRDNAKNTLYLQMNSLRAEDTAVYYCARHRYNLFDSWGQGTLVTVSS

SEQ ID NO: 14 - protein, 117 aa, Artificial sequence
  Humanised heavy chain variable region
EVQLVESGGGLVQPGRSLRLSCAASGFIFSEHNMAWVRQAPGKGLEWVSTISDDGRNTYYRDSMRGRFTISRDNAKNSLYLQMNSLRAEDTALYYCAKHRYNLFDSWGQGTLVTVSS

SEQ ID NO: 15 - protein, 26 aa, Rattus norvegicus
DIQMTQSPSFLSASVGDRVTINCKAS

SEQ ID NO: 16 - protein, 6 aa, Rattus norvegicus
QNIDRY

SEQ ID NO: 17 - protein, 17 aa, Rattus norvegicus
LNWYQQKLGEAPKRLLY

SEQ ID NO: 18 - protein, 3 aa, Rattus norvegicus
NTN

SEQ ID NO: 19 - protein, 36 aa, Rattus norvegicus
KLQTGIPSRFSGSGSATDFTLTISSLQPEDFATYFC

SEQ ID NO: 20 - protein, 9 aa, Rattus norvegicus
LQYNSLPLT

SEQ ID NO: 21 - protein, 10 aa, Rattus norvegicus
FGSGTKLEIK

SEQ ID NO: 22 - protein, 25 aa, Rattus norvegicus
EVQLVESGGGLVQPGRSLKLSCAAS

SEQ ID NO: 23 - protein, 8 aa, Rattus norvegicus
GFIFSEHN

SEQ ID NO: 24 - protein, 17 aa, Rattus norvegicus
MAWVRQAPKKGLEWVAT

SEQ ID NO: 25 - protein, 8 aa, Rattus norvegicus
ISDDGRNT

SEQ ID NO: 26 - protein, 38 aa, Rattus norvegicus
YYRDSMRGRFTISRENARSTLYLQLDSLRSEDTATYYC

SEQ ID NO: 27 - protein, 10 aa, Rattus norvegicus
ASHRYNLFDS

SEQ ID NO: 28 - protein, 11 aa, Rattus norvegicus
WGQGVMVTVSS

SEQ ID NO: 29 - protein, 26 aa, Homo sapiens [sequence omitted]

SEQ ID NO: 30 - protein, 17 aa, Homo sapiens
LNWYQQKPGKAPKRLIY

SEQ ID NO: 31 - protein, 36 aa, Homo sapiens
KLQTGVPSRFSGSGSGTEFTLTISSLQPEDFATYYC

SEQ ID NO: 32 - protein, 10 aa, Homo sapiens
FGQGTKLEIK

SEQ ID NO: 33 - protein, 25 aa, Homo sapiens
QVQLVESGGGVVQPGRSLRLSCAAS

SEQ ID NO: 34 - protein, 17 aa, Homo sapiens
MAWVRQAPGKGLEWVAT

SEQ ID NO: 35 - protein, 40 aa, Homo sapiens
YYRDSMRGRFTISRDNSKNTLYLQMNSLRAEDTAVYYCTS

SEQ ID NO: 36 - protein, 10 aa, Artificial sequence
  Humanised heavy chain CDR3
TSHRYNLFDS

SEQ ID NO: 37 - protein, 11 aa, Homo sapiens
WGQGTMVTVSS

SEQ ID NO: 38 - protein, 17 aa, Homo sapiens
LNWFQQKPGKAPKSLIY

SEQ ID NO: 39 - protein, 36 aa, Homo sapiens
KLQTGVPSKFSGSGSGTDFTLTISSLQPEDFATYYC

SEQ ID NO: 40 - protein, 10 aa, Homo sapiens
FGQGTRLEIK

SEQ ID NO: 41 - protein, 25 aa, Homo sapiens [sequence omitted]

SEQ ID NO: 42 - protein, 17 aa, Homo sapiens
MAWVRQAPGKGLEWVST

SEQ ID NO: 43 - protein, 40 aa, Homo sapiens
YYRDSMRGRFTISRDNSKNTLYLQMNSLRAEDTAVYYCAK

SEQ ID NO: 44 - protein, 10 aa, Artificial sequence
  Humanised heavy chain CDR3
AKHRYNLFDS

SEQ ID NO: 45 - protein, 11 aa, Homo sapiens
WGQGTLVTVSS

SEQ ID NO: 46 - protein, 17 aa, Homo sapiens
LNWYQQKPGKAPKLLIY

SEQ ID NO: 47 - protein, 36 aa, Homo sapiens
KLQTGVPSRFSGSGSGTDFTLTISSLQPEDFATYYC

SEQ ID NO: 48 - protein, 40 aa, Homo sapiens
YYRDSMRGRFTISRDNAKNSLYLQMNSLRAEDTAVYYCAR

SEQ ID NO: 49 - protein, 10 aa, Artificial sequence
  Humanised heavy chain CDR3
ARHRYNLFDS

SEQ ID NO: 50 - protein, 26 aa, Homo sapiens
DIQLTQSPSFLSASVGDRVTITCKAS

SEQ ID NO: 51 - protein, 17 aa, Homo sapiens
MAWVRQAPGKGLVWVST

SEQ ID NO: 52 - protein, 40 aa, Homo sapiens
YYRDSMRGRFTISRDNAKNTLYLQMNSLRAEDTAVYYCAR

SEQ ID NO: 53 - protein, 26 aa, Homo sapiens
DIQMTQSPSTLSASVGDRVTITCKAS

SEQ ID NO: 54 - protein, 36 aa, Homo sapiens
KLQTGVPSRFSGSGSGTEFTLTISSLQPDDFATYYC

SEQ ID NO: 55 - protein, 25 aa, Homo sapiens [sequence omitted]

SEQ ID NO: 56 - protein, 40 aa, Homo sapiens
YYRDSMRGRFTISRDNAKNSLYLQMNSLRAEDTALYYCAK

SEQ ID NO: 57 - protein, 10 aa, Artificial sequence
  Heavy chain CDR3
  misc_feature (1)..(1): Xaa can be Ala or Thr
  misc_feature (2)..(2): Xaa can be Ser, Lys or Arg
XXHRYNLFDS

SEQ ID NO: 58 - protein, 11 aa, Rattus norvegicus
KASQNIDRYLN

SEQ ID NO: 59 - protein, 7 aa, Rattus norvegicus
NTNKLQT

SEQ ID NO: 60 - protein, 5 aa, Rattus norvegicus
EHNMA

SEQ ID NO: 61 - protein, 17 aa, Rattus norvegicus
TISDDGRNTYYRDSMRG

SEQ ID NO: 62 - protein, 8 aa, Rattus norvegicus
HRYNLFDS